European Patent Application EP 4 032 907 A9, published January 4, 2023. Title: BCMA-TARGETED ANTIBODY AND CHIMERIC ANTIGEN RECEPTOR. Applicant: SHANGHAI GENBASE BIOTECHNOLOGY CO., LTD. The sequence listing filed with the application follows.

SEQUENCE LISTING (16 sequences)

SEQ ID NO: 1 - protein, 117 aa, Artificial sequence
  C11D5.3-03 VH
QIQLVQSGSELKKPGASVKVSCKASGYTFTDYSINWVRQAPGQGLEWMGWINTETREPAYAQGFTGRFVFSLDTSVSTAYLQISSLKAEDTAVYFCALDYSYAMDYWGQGTLVTVSS

SEQ ID NO: 2 - protein, 111 aa, Artificial sequence
  C11D5.3-03 VL
EIVLTQSPATLSMSLGERATLSCRASQSVTILGSHLIHWYQQKPGQPPRLLIQLASNVQTGIPARFSGSGSRTDFTLTISSLEEEDFAVYYCLQSRTIPRTFGGGTKVEIK

SEQ ID NO: 3 - protein, 117 aa, Artificial sequence
  C11D5.3-04 VH
QIQLVQSGSELKKPGASVKVSCKASGYTFTDYSMNWVRQAPGQGLEWMGWINTETREPTYAQGFTGRFVFSLDTSVSTAYLQISSLKAEDTAVYFCALDYSYAMDYWGQGTLVTVSS

SEQ ID NO: 4 - protein, 111 aa, Artificial sequence
  C11D5.3-04 VL
EIVLTQSPATLSMSLGERATLSCRASESVTILGSHLIHWYQQKPGQPPRLLIQLASNRATGIPARFSGSGSRTDFTLTISSLEEEDFAVYYCLQSRTIPRTFGGGTKVEIK

SEQ ID NO: 5 - protein, 15 aa, Artificial sequence
  Linker
GGGGSGGGGSGGGGS

SEQ ID NO: 6 - protein, 45 aa, Artificial sequence
  Hinge region
TTTPAPRPPTPAPTIASQPLSLRPEACRPAAGGAVHTRGLDFACD

SEQ ID NO: 7 - protein, 24 aa, Artificial sequence
  Transmembrane region
IYIWAPLAGTCGVLLLSLVITLYC

SEQ ID NO: 8 - protein, 41 aa, Artificial sequence
  CD137 intracellular signaling domain
KRGRKKLLYIFKQPFMRPVQTTQEEDGCSCRFPEEEEGGCE

SEQ ID NO: 9 - protein, 113 aa, Artificial sequence
  CD3(Zeta)ITAM
LRVKFSRSADAPAYKQGQNQLYNELNLGRREEYDVLDKRRGRDPEMGGKPRRKNPQEGLYNELQKDKMAEAYSEIGMKGERRRGKGHDGLYQGLSTATKDTYDALHMQALPPR

SEQ ID NO: 10 - protein, 466 aa, Artificial sequence
  C11D5.3-03-CAR full-length amino acid sequence
QIQLVQSGSELKKPGASVKVSCKASGYTFTDYSINWVRQAPGQGLEWMGWINTETREPAYAQGFTGRFVFSLDTSVSTAYLQISSLKAEDTAVYFCALDYSYAMDYWGQGTLVTVSSGGGGSGGGGSGGGGSEIVLTQSPATLSMSLGERATLSCRASQSVTILGSHLIHWYQQKPGQPPRLLIQLASNVQTGIPARFSGSGSRTDFTLTISSLEEEDFAVYYCLQSRTIPRTFGGGTKVEIKTTTPAPRPPTPAPTIASQPLSLRPEACRPAAGGAVHTRGLDFACDIYIWAPLAGTCGVLLLSLVITLYCKRGRKKLLYIFKQPFMRPVQTTQEEDGCSCRFPEEEEGGCELRVKFSRSADAPAYKQGQNQLYNELNLGRREEYDVLDKRRGRDPEMGGKPRRKNPQEGLYNELQKDKMAEAYSEIGMKGERRRGKGHDGLYQGLSTATKDTYDALHMQALPPR

SEQ ID NO: 11 - DNA, 1398 bp, Artificial sequence
  Nucleic acid sequence encoding C11D5.3-03-CAR
cagatccagctggtgcaatctgggtctgagttgaagaagcctggggcctcagtgaaggtttcctgcaaggcttctggatacaccttcactgattattccatcaattgggtgcgccaggcccctggacaagggcttgagtggatgggatggatcaacaccgaaactagggagccagcctatgcccagggcttcacaggacggtttgtcttctccttggacacctctgtcagcacggcatatctgcagatcagcagcctaaaggctgaggacactgccgtgtatttctgtgcgctggattatagctatgctatggactactggggccagggaaccctggtcaccgtctccagcggtggaggtggcagcggaggaggtgggtccggcggtggaggaagcgaaattgtgttgacacagtctccagccaccctgtctatgtctctgggggaaagagccaccctctcctgcagggccagtcagagtgttaccatccttggtagccaccttatacactggtaccaacagaaacctggccagcctcccaggctcctcatccaattggcatccaacgtgcaaactggcatcccagccaggttcagtggcagtgggtctaggacagacttcactctcaccatcagcagcctagaggaggaagattttgcagtttattactgtctgcagagtagaactattccacggactttcggcggagggaccaaggtggagatcaaaaccacgacgccagcgccgcgaccaccaacaccggcgcccaccatcgcgtcgcagcccctgtccctgcgcccagaggcgtgccggccagcggcggggggcgcagtgcacacgagggggctggacttcgcctgtgatatctacatctgggcgcccttggccgggacttgtggggtccttctcctgtcactggttatcaccctttactgcaaacggggcagaaagaaactcctgtatatattcaaacaaccatttatgagaccagtacaaactactcaagaggaagatggctgtagctgccgatttccagaagaagaagaaggaggatgtgaactgagagtgaagttcagcaggagcgcagacgcccccgcgtacaagcagggccagaaccagctctataacgagctcaatctaggacgaagagaggagtacgatgttttggacaagagacgtggccgggaccctgagatggggggaaagccgagaaggaagaaccctcaggaaggcctgtacaatgaactgcagaaagataagatggcggaggcctacagtgagattgggatgaaaggcgagcgccggaggggcaaggggcacgatggcctttaccagggtctcagtacagccaccaaggacacctacgacgcccttcacatgcaggccctgccccctcgc

SEQ ID NO: 12 - protein, 466 aa, Artificial sequence
  C11D5.3-04-CAR full-length amino acid sequence
QIQLVQSGSELKKPGASVKVSCKASGYTFTDYSMNWVRQAPGQGLEWMGWINTETREPTYAQGFTGRFVFSLDTSVSTAYLQISSLKAEDTAVYFCALDYSYAMDYWGQGTLVTVSSGGGGSGGGGSGGGGSEIVLTQSPATLSMSLGERATLSCRASESVTILGSHLIHWYQQKPGQPPRLLIQLASNRATGIPARFSGSGSRTDFTLTISSLEEEDFAVYYCLQSRTIPRTFGGGTKVEIKTTTPAPRPPTPAPTIASQPLSLRPEACRPAAGGAVHTRGLDFACDIYIWAPLAGTCGVLLLSLVITLYCKRGRKKLLYIFKQPFMRPVQTTQEEDGCSCRFPEEEEGGCELRVKFSRSADAPAYKQGQNQLYNELNLGRREEYDVLDKRRGRDPEMGGKPRRKNPQEGLYNELQKDKMAEAYSEIGMKGERRRGKGHDGLYQGLSTATKDTYDALHMQALPPR

SEQ ID NO: 13 - DNA, 1398 bp, Artificial sequence
  Nucleic acid sequence encoding C11D5.3-04-CAR
cagatccagctggtgcaatctgggtctgagttgaagaagcctggggcctcagtgaaggtttcctgcaaggcttctggatacaccttcactgattattccatgaattgggtgcgccaggcccctggacaagggcttgagtggatgggatggatcaacaccgaaactagggagccaacgtatgcccagggcttcacaggacggtttgtcttctccttggacacctctgtcagcacggcatatctgcagatcagcagcctaaaggctgaggacactgccgtgtatttctgtgcgctggattatagctatgctatggactactggggccagggaaccctggtcaccgtctccagcggtggaggtggcagcggaggaggtgggtccggcggtggaggaagcgaaattgtgttgacacagtctccagccaccctgtctatgtctctgggggaaagagccaccctctcctgcagggccagtgagagtgttaccatccttggtagccaccttatacactggtaccaacagaaacctggccagcctcccaggctcctcatccaattggcatccaacagggccactggcatcccagccaggttcagtggcagtgggtctaggacagacttcactctcaccatcagcagcctagaggaggaagattttgcagtttattactgtctgcagagtagaactattccacggactttcggcggagggaccaaggtggagatcaaaaccacgacgccagcgccgcgaccaccaacaccggcgcccaccatcgcgtcgcagcccctgtccctgcgcccagaggcgtgccggccagcggcggggggcgcagtgcacacgagggggctggacttcgcctgtgatatctacatctgggcgcccttggccgggacttgtggggtccttctcctgtcactggttatcaccctttactgcaaacggggcagaaagaaactcctgtatatattcaaacaaccatttatgagaccagtacaaactactcaagaggaagatggctgtagctgccgatttccagaagaagaagaaggaggatgtgaactgagagtgaagttcagcaggagcgcagacgcccccgcgtacaagcagggccagaaccagctctataacgagctcaatctaggacgaagagaggagtacgatgttttggacaagagacgtggccgggaccctgagatggggggaaagccgagaaggaagaaccctcaggaaggcctgtacaatgaactgcagaaagataagatggcggaggcctacagtgagattgggatgaaaggcgagcgccggaggggcaaggggcacgatggcctttaccagggtctcagtacagccaccaaggacacctacgacgcccttcacatgcaggccctgccccctcgc

SEQ ID NO: 14 - protein, 466 aa, Artificial sequence
  C11D5.3-CAR full-length amino acid sequence
QIQLVQSGPELKKPGETVKISCKASGYTFTDYSINWVKRAPGKGLKWMGWINTETREPAYAYDFRGRFAFSLETSASTAYLQINNLKYEDTATYFCALDYSYAMDYWGQGTSVTVSSGGGGSGGGGSGGGGSDIVLTQSPPSLAMSLGKRATISCRASESVTILGSHLIHWYQQKPGQPPTLLIQLASNVQTGVPARFSGSGSRTDFTLTIDPVEEDDVAVYYCLQSRTIPRTFGGGTKLEIKTTTPAPRPPTPAPTIASQPLSLRPEACRPAAGGAVHTRGLDFACDIYIWAPLAGTCGVLLLSLVITLYCKRGRKKLLYIFKQPFMRPVQTTQEEDGCSCRFPEEEEGGCELRVKFSRSADAPAYKQGQNQLYNELNLGRREEYDVLDKRRGRDPEMGGKPRRKNPQEGLYNELQKDKMAEAYSEIGMKGERRRGKGHDGLYQGLSTATKDTYDALHMQALPPR

SEQ ID NO: 15 - DNA, 1398 bp, Artificial sequence
  Nucleic acid sequence encoding C11D5.3-CAR
cagatccagctggtgcaatctgggccagagttgaagaagcctggggagaccgtgaagatctcctgcaaggcttctggatacaccttcactgattattccatcaattgggtgaagcgggcccctggaaaggggcttaagtggatgggatggatcaacaccgaaactagggagccagcctatgcctacgacttcaggggacggtttgccttctccttggaaacctctgcgagcacggcatatctgcagatcaacaacctaaagtatgaggacactgccacatatttctgtgcgttagactacagttacgctatggactactggggccaagggacctcggtcaccgtctccagcggtggaggtggcagcggaggaggtgggtccggcggtggaggaagcgacattgtgctgacccagtctccaccctccttggccatgtctctgggaaagagggccaccatctcctgcagagccagcgagagtgtcaccatcttgggaagccacttaattcactggtatcagcagaaaccaggacaacctcctaccctcctgattcaattggcatccaatgtgcaaactggggtcccagccaggttcagcggcagtgggtctaggaccgatttcaccctcacaattgaccctgtggaagaggatgatgtggcagtttattactgtctgcagagtagaactattcctcggacttttggcggagggaccaagctggagatcaaaaccacgacgccagcgccgcgaccaccaacaccggcgcccaccatcgcgtcgcagcccctgtccctgcgcccagaggcgtgccggccagcggcggggggcgcagtgcacacgagggggctggacttcgcctgtgatatctacatctgggcgcccttggccgggacttgtggggtccttctcctgtcactggttatcaccctttactgcaaacggggcagaaagaaactcctgtatatattcaaacaaccatttatgagaccagtacaaactactcaagaggaagatggctgtagctgccgatttccagaagaagaagaaggaggatgtgaactgagagtgaagttcagcaggagcgcagacgcccccgcgtacaagcagggccagaaccagctctataacgagctcaatctaggacgaagagaggagtacgatgttttggacaagagacgtggccgggaccctgagatggggggaaagccgagaaggaagaaccctcaggaaggcctgtacaatgaactgcagaaagataagatggcggaggcctacagtgagattgggatgaaaggcgagcgccggaggggcaaggggcacgatggcctttaccagggtctcagtacagccaccaaggacacctacgacgcccttcacatgcaggccctgccccctcgc

SEQ ID NO: 16 - DNA, 1128 bp, Artificial sequence
  Nucleic acid sequence encoding P2A-tEGFR
gccaccaacttcagcctgctgaagcaggccggcgacgtggaggagaaccccggccccatgcttctcctggtgacaagccttctgctctgtgagttaccacacccagcattcctcctgatcccacgcaaagtgtgtaacggaataggtattggtgaatttaaagactcactctccataaatgctacgaatattaaacacttcaaaaactgcacctccatcagtggcgatctccacatcctgccggtggcatttaggggtgactccttcacacatactcctcctctggatccacaggaactggatattctgaaaaccgtaaaggaaatcacagggtttttgctgattcaggcttggcctgaaaacaggacggacctccatgcctttgagaacctagaaatcatacgcggcaggaccaagcaacatggtcagttttctcttgcagtcgtcagcctgaacataacatccttgggattacgctccctcaaggagataagtgatggagatgtgataatttcaggaaacaaaaatttgtgctatgcaaatacaataaactggaaaaaactgtttgggacctccggtcagaaaaccaaaattataagcaacagaggtgaaaacagctgcaaggccacaggccaggtctgccatgccttgtgctcccccgagggctgctggggcccggagcccagggactgcgtctcttgccggaatgtcagccgaggcagggaatgcgtggacaagtgcaaccttctggagggtgagccaagggagtttgtggagaactctgagtgcatacagtgccacccagagtgcctgcctcaggccatgaacatcacctgcacaggacggggaccagacaactgtatccagtgtgcccactacattgacggcccccactgcgtcaagacctgcccggcaggagtcatgggagaaaacaacaccctggtctggaagtacgcagacgccggccatgtgtgccacctgtgccatccaaactgcacctacggatgcactgggccaggtcttgaaggctgtccaacgaatgggcctaagatcccgtccatcgccactgggatggtgggggccctcctcttgctgctggtggtggccctggggatcggcctcttcatg